European Patent Specification EP 3 645 552 B1, published June 28, 2023. Title: NOVEL PROTEIN PORES. Applicant: VIB VZW VRIJE UNIVERSITEIT BRUSSEL OXFORD NANOPORE TECHNOLOGIES LIMITED. The sequence listing filed with the application follows.

SEQUENCE LISTING (120 sequences)

SEQ ID NO: 1 - DNA, 834 bp, Escherichia coli
atgcagcgcttatttcttttggttgccgtcatgttactgagcggatgcttaaccgccccgcctaaagaagccgccagaccgacattaatgcctcgtgctcagagctacaaagatttgacccatctgccagcgccgacgggtaaaatctttgtttcggtatacaacattcaggacgaaaccgggcaatttaaaccctacccggcaagtaacttctccactgctgttccgcaaagcgccacggcaatgctggtcacggcactgaaagattctcgctggtttataccgctggagcgccagggcttacaaaacctgcttaacgagcgcaagattattcgtgcggcacaagaaaacggcacggttgccattaataaccgaatcccgctgcaatctttaacggcggcaaatatcatggttgaaggttcgattatcggttatgaaagcaacgtcaaatctggcggggttggggcaagatattttggcatcggtgccgacacgcaataccagctcgatcagattgccgtgaacctgcgcgtcgtcaatgtgagtaccggcgagatcctttcttcggtgaacaccagtaagacgatactttcctatgaagttcaggccggggttttccgctttattgactaccagcgcttgcttgaaggggaagtgggttacacctcgaacgaacctgttatgctgtgcctgatgtcggctatcgaaacaggggtcattttcctgattaatgatggtatcgaccgtggtctgtgggatttgcaaaataaagcagaacggcagaatgacattctggtgaaataccgccatatgtcggttccaccggaatcctga

SEQ ID NO: 2 - protein, 277 aa, Escherichia coli
MQRLFLLVAVMLLSGCLTAPPKEAARPTLMPRAQSYKDLTHLPAPTGKIFVSVYNIQDETGQFKPYPASNFSTAVPQSATAMLVTALKDSRWFIPLERQGLQNLLNERKIIRAAQENGTVAINNRIPLQSLTAANIMVEGSIIGYESNVKSGGVGARYFGIGADTQYQLDQIAVNLRVVNVSTGEILSSVNTSKTILSYEVQAGVFRFIDYQRLLEGEVGYTSNEPVMLCLMSAIETGVIFLINDGIDRGLWDLQNKAERQNDILVKYRHMSVPPES

SEQ ID NO: 3 - protein, 262 aa, Escherichia coli
CLTAPPKEAARPTLMPRAQSYKDLTHLPAPTGKIFVSVYNIQDETGQFKPYPASNFSTAVPQSATAMLVTALKDSRWFIPLERQGLQNLLNERKIIRAAQENGTVAINNRIPLQSLTAANIMVEGSIIGYESNVKSGGVGARYFGIGADTQYQLDQIAVNLRVVNVSTGEILSSVNTSKTILSYEVQAGVFRFIDYQRLLEGEVGYTSNEPVMLCLMSAIETGVIFLINDGIDRGLWDLQNKAERQNDILVKYRHMSVPPES

SEQ ID NO: 4 - protein, 414 aa, Escherichia coli
ATGCGTGTCAAACATGCAGTAGTTCTACTCATGCTTATTTCGCCATTAAGTTGGGCTGGAACCATGACTTTCCAGTTCCGTAATCCAAACTTTGGTGGTAACCCAAATAATGGCGCTTTTTTATTAAATAGCGCTCAGGCCCAAAACTCTTATAAAGATCCGAGCTATAACGATGACTTTGGTATTGAAACACCCTCAGCGTTAGATAACTTTACTCAGGCCATCCAGTCACAAATTTTAGGTGGGCTACTGTCGAATATTAATACCGGTAAACCGGGCCGCATGGTGACCAACGATTATATTGTCGATATTGCCAACCGCGATGGTCAATTGCAGTTGAACGTGACAGATCGTAAAACCGGACAAACCTCGACCATCCAGGTTTCGGGTTTACAAAATAACTCAACCGATTTT

SEQ ID NO: 5 - protein, 138 aa, Escherichia coli
MRVKHAVVLLMLISPLSWAGTMTFQFRNPNFGGNPNNGAFLLNSAQAQNSYKDPSYNDDFGIETPSALDNFTQAIQSQILGGLLSNINTGKPGRMVTNDYIVDIANRDGQLQLNVTDRKTGQTSTIQVSGLQNNSTDF

SEQ ID NO: 6 - protein, 119 aa, Escherichia coli
GTMTFQFRNPNFGGNPNNGAFLLNSAQAQNSYKDPSYNDDFGIETPSALDNFTQAIQSQILGGLLSNINTGKPGRMVTNDYIVDIANRDGQLQLNVTDRKTGQTSTIQVSGLQNNSTDF

SEQ ID NO: 7 - DNA, 106 bp, Artificial Sequence
  fragment of wild-type E. coli CsgF encoding amino acids 1 to 27 and a C-terminal 6 His tag
atgcgtgtcaaacatgcagtagttctactcatgcttatttcgccattaagttgggctggaaccatgactttccagttccgtcatcaccatcaccatcactaagccc

SEQ ID NO: 8 - protein, 33 aa, Artificial Sequence
  fragment of wild-type E. coli CsgF encompassing amino acids 1 to 27 and a C-terminal 6 His tag
MRVKHAVVLLMLISPLSWAGTMTFQFRHHHHHH

SEQ ID NO: 9 - DNA, 139 bp, Artificial Sequence
  fragment of wild-type E. coli CsgF encoding amino acids 1 to 38 and a C-terminal 6 His tag
atgcgtgtcaaacatgcagtagttctactcatgcttatttcgccattaagttgggctggaaccatgactttccagttccgtaatccaaactttggtggtaacccaaataatggccatcaccatcaccatcactaagccc

SEQ ID NO: 10 - protein, 44 aa, Artificial Sequence
  fragment of wild-type E. coli CsgF encompassing amino acids 1 to 38 and a C-terminal 6 His tag
MRVKHAVVLLMLISPLSWAGTMTFQFRNPNFGGNPNNGHHHHHH

SEQ ID NO: 11 - DNA, 169 bp, Artificial Sequence
  fragment of wild-type E. coli CsgF encoding amino acids 1 to 48 and a C-terminal 6 His tag
atgcgtgtcaaacatgcagtagttctactcatgcttatttcgccattaagttgggctggaaccatgactttccagttccgtaatccaaactttggtggtaacccaaataatggcgcttttttattaaatagcgctcaggcccaacatcaccatcaccatcactaagccc

SEQ ID NO: 12 - protein, 54 aa, Artificial Sequence
  fragment of wild-type E. coli CsgF encompassing amino acids 1 to 48 and a C-terminal 6 His tag
MRVKHAVVLLMLISPLSWAGTMTFQFRNPNFGGNPNNGAFLLNSAQAQHHHHHH

SEQ ID NO: 13 - DNA, 217 bp, Artificial Sequence
  fragment of wild-type E. coli CsgF encoding amino acids 1 to 64 and a C-terminal 6 His tag
atgcgtgtcaaacatgcagtagttctactcatgcttatttcgccattaagttgggctggaaccatgactttccagttccgtaatccaaactttggtggtaacccaaataatggcgcttttttattaaatagcgctcaggcccaaaactcttataaagatccgagctataacgatgactttggtattgaaacacatcaccatcaccatcactaagccc

SEQ ID NO: 14 - protein, 70 aa, Artificial Sequence
  fragment of wild-type E. coli CsgF encompassing amino acids 1 to 64 and a C-terminal 6 His tag
MRVKHAVVLLMLISPLSWAGTMTFQFRNPNFGGNPNNGAFLLNSAQAQNSYKDPSYNDDFGIETHHHHHH

SEQ ID NO: 15 - protein, 34 aa, Artificial Sequence
  residues 20 to 53 of E. coli CsgF
GTMTFQFRNPNFGGNPNNGAFLLNSAQAQNSYKD

SEQ ID NO: 16 - protein, 25 aa, Artificial Sequence
  residues 20 to 42 of E. coli CsgF, including KD at its C-terminus
GTMTFQFRNPNFGGNPNNGAFLLKD

SEQ ID NO: 17 - protein, 32 aa, Artificial Sequence
  residues 23 to 55 of CsgF homologue Q88H88
TELVYTPVNPAFGGNPLNGTWLLNNAQAQNDY

SEQ ID NO: 18 - protein, 32 aa, Artificial Sequence
  residues 25 to 57 of CsgF homologue A0A143HJA0
TELIYEPVNPNFGGNPLNGSYLLNNAQAQDRH

SEQ ID NO: 19 - protein, 32 aa, Artificial Sequence
  residues 21 to 53 of CsgF homologue Q5E245
SELVYTPVNPNFGGNPLNTSHLFGGANAINDY

SEQ ID NO: 20 - protein, 32 aa, Artificial Sequence
  residues 19 to 51 of CsgF homologue Q084E5
TQLVYTPVNPAFGGSYLNGSYLLANASAQNEH

SEQ ID NO: 21 - protein, 32 aa, Artificial Sequence
  residues 15 to 47 of CsgF homologue F0LZU2
SSLVYEPVNPTFGGNPLNTTHLFSRAEAINDY

SEQ ID NO: 22 - protein, 32 aa, Artificial Sequence
  residues 26 to 58 of CsgF homologue A0A136HQR0
TELVYEPINPSFGGNPLNGSFLLSKANSQNAH

SEQ ID NO: 23 - protein, 32 aa, Artificial Sequence
  residues 21 to 53 of CsgF homologue A0A0W1SRL3
TEIVYQPINPSFGGNPMNGSFLLQKAQSQNAH

SEQ ID NO: 24 - protein, 33 aa, Artificial Sequence
  residues 26 to 59 of CsgF homologue B0UH01
SSLVYQPVNPAFGGPQLNGSWLQAEANAQNIPQ

SEQ ID NO: 25 - protein, 31 aa, Artificial Sequence
  residues 22 to 53 of CsgF homologue Q6NAU5
GSLVYTPTNPAFGGSPLNGSWQMQQATAGNH

SEQ ID NO: 26 - protein, 32 aa, Artificial Sequence
  residues 7 to 38 of CsgF homologue G8PUY5
QQLIYQPTNPSFGGYAANTTHLFATANAQKTA

SEQ ID NO: 27 - protein, 32 aa, Artificial Sequence
  residues 25 to 57 of CsgF homologue A0A0S2ETP7
GDLVYTPVNPSFGGSPLNSAHLLSIAGAQKNA

SEQ ID NO: 28 - protein, 32 aa, Artificial Sequence
  residues 19 to 51 of CsgF homologue E3I1Z1
AELGYTPVNPSFGGSPLNGSTLLSEASAQKPN

SEQ ID NO: 29 - protein, 31 aa, Artificial Sequence
  residues 24 to 55 of CsgF homologue F3Z094
TELVFSFTNPSFGGDPMIGNFLLNKADSQKR

SEQ ID NO: 30 - protein, 32 aa, Artificial Sequence
  residues 21 to 53 of CsgF homologue A0A176T7M2
QQLVYKSINPFFGGGDSFAYQQLLASANAQND

SEQ ID NO: 31 - protein, 31 aa, Artificial Sequence
  residues 14 to 45 of CsgF homologue D2QPP8
QALVYHPNNPAFGGNTFNYQWMLSSAQAQDR

SEQ ID NO: 32 - protein, 32 aa, Artificial Sequence
  residues 28 to 58 of CsgF homologue N2IYT1
TELVYTPKNPAFGGSPLNGSYLLGNAQAQNDY

SEQ ID NO: 33 - protein, 32 aa, Artificial Sequence
  residues 26 to 58 of CsgF homologue W7QHV5
GQLIYQPINPSFGGDPLLGNHLLNKAQAQDTK

SEQ ID NO: 34 - protein, 32 aa, Artificial Sequence
  residues 23 to 55 of CsgF homologue D4ZLW2
TQLIYTPVNPNFGGSYLNGSYLLANASVQNDH

SEQ ID NO: 35 - protein, 32 aa, Artificial Sequence
  residues 21 to 53 of CsgF homologue D2QT92
QAFVYHPNNPNFGGNTFNYSWMLSSAQAQDRT

SEQ ID NO: 36 - protein, 31 aa, Artificial Sequence
  residues 20 to 51 of CsgF homologue A0A167UJA2
QGLIYKPKNPAFGGDTFNYQWLASSAESQNK

SEQ ID NO: 37 - protein, 8 aa, Artificial Sequence
  residues 20 to 27 of wild-type E. coli CsgF
GTMTFQFR

SEQ ID NO: 38 - protein, 19 aa, Artificial Sequence
  residues 20 to 38 of wild-type E. coli CsgF
GTMTFQFRNPNFGGNPNNG

SEQ ID NO: 39 - protein, 29 aa, Artificial Sequence
  residues 20 to 48 of wild-type E. coli CsgF
GTMTFQFRNPNFGGNPNNGAFLLNSAQAQ

SEQ ID NO: 40 - protein, 45 aa, Artificial Sequence
  residues 20 to 64 of wild-type E. coli CsgF
GTMTFQFRNPNFGGNPNNGAFLLNSAQAQNSYKDPSYNDDFGIET

SEQ ID NO: 41 - DNA, 24 bp, Artificial Sequence
  primer CsgF_d27_end
acggaactggaaagtcatggttcc

SEQ ID NO: 42 - DNA, 30 bp, Artificial Sequence
  primer CsgF_d38_end
gccattatttgggttaccaccaaagtttgg

SEQ ID NO: 43 - DNA, 30 bp, Artificial Sequence
  primer CsgF_d48_end
ttgggcctgagcgctatttaataaaaaagc

SEQ ID NO: 44 - DNA, 33 bp, Artificial Sequence
  primer CsgF_d64_end
tgtttcaataccaaagtcatcgttatagctcgg

SEQ ID NO: 45 - DNA, 25 bp, Artificial Sequence
  primer pNa62_CsgF_histag_Fw
catcaccatcaccatcactaagccc

SEQ ID NO: 46 - DNA, 32 bp, Artificial Sequence
  primer CsgF-His_pET22b_FW
cccccatatgggaaccatgactttccagttcc

SEQ ID NO: 47 - DNA, 55 bp, Artificial Sequence
  primer CsgF-His_pET22b_Rev
ccccgaattcctaatggtgatggtgatggtggtaaaaatcggttgagttattttg

SEQ ID NO: 48 - DNA, 58 bp, Artificial Sequence
  primer csgEFG_pDONR221_FW
ggggacaagtttgtacaaaaaagcaggctacctcaggcgataaagccatgaaacgtta

SEQ ID NO: 49 - DNA, 72 bp, Artificial Sequence
  primer csgEFG_pDONR221_Rev
ggggaccactttgtacaagaaagctgggtgtttaaactcatttttcgaactgcgggtggctccaagcgctgg

SEQ ID NO: 50 - DNA, 59 bp, Artificial Sequence
  primer Mut_csgF_His_FW
caaaataactcaaccgattttcatcaccatcaccatcactaagccccagcttcataagg

SEQ ID NO: 51 - DNA, 59 bp, Artificial Sequence
  primer Mut_csgF_His_Rev
ccttatgaagctggggcttagtgatggtgatggtgatgaaaatcggttgagttattttg

SEQ ID NO: 52 - DNA, 21 bp, Artificial Sequence
  primer DelCsgE_Rev
agcctgcttttttgtacaaac

SEQ ID NO: 53 - DNA, 23 bp, Artificial Sequence
  primer DelCsgE FW
ataaaaaattgttcggaggctgc

SEQ ID NO: 54 - protein, 30 aa, Artificial Sequence
  residues 1 to 29 of mature E. coli CsgF
GTMTFQFRNPNFGGNPNNGAFLLNSAQAQN

SEQ ID NO: 55 - protein, 35 aa, Artificial Sequence
  residues 1 to 45 of mature E. coli CsgF
GTMTFQFRNPNFGGNPNNGAFLLNSAQAQNSYKDP

SEQ ID NO: 56 - protein, 155 aa, Artificial Sequence
  a mutated (T4C/N17S) CsgF sequence with a signal sequence, and a TEV protease cleavage site (ENLYFQS) inserted between residues 35 and 36 of sequence of the mature protein
MRVKHAVVLLMLISPLSWAGTMCFQFRNPNFGGNPSNGAFLLNSAQAQNSYKDPENLYFQSSYNDDFGIETPSALDNFTQAIQSQILGGLLSNINTGKPGRMVTNDYIVDIANRDGQLQLNVTDRKTGQTSTIQVSGLQNNSTDFSAWSHPQFEK

SEQ ID NO: 57 - protein, 155 aa, Artificial Sequence
  a mutated (N17S-Del) CsgF sequence with a signal sequence, and a TEV protease cleavage site (ENLYFQS) inserted between residues 35 and 36 of sequence of the mature protein
MRVKHAVVLLMLISPLSWAGTMTFQFRNPNFGGNPSNGAFLLNSAQAQNSYKDPENLYFQSSYNDDFGIETPSALDNFTQAIQSQILGGLLSNINTGKPGRMVTNDYIVDIANRDGQLQLNVTDRKTGQTSTIQVSGLQNNSTDFSAWSHPQFEK

SEQ ID NO: 58 - protein, 155 aa, Artificial Sequence
  a mutated (G1C/N17S) CsgF sequence with a signal sequence, and a TEV protease cleavage site (ENLYFQS) inserted between residues 35 and 36 of sequence of the mature protein
MRVKHAVVLLMLISPLSWACTMTFQFRNPNFGGNPSNGAFLLNSAQAQNSYKDPENLYFQSSYNDDFGIETPSALDNFTQAIQSQILGGLLSNINTGKPGRMVTNDYIVDIANRDGQLQLNVTDRKTGQTSTIQVSGLQNNSTDFSAWSHPQFEK

SEQ ID NO: 59 - protein, 155 aa, Artificial Sequence
  a mutated (G1C) CsgF sequence with a signal sequence, and a TEV protease cleavage site (ENLYFQS) inserted between residues 35 and 36 of sequence of the mature protein
MRVKHAVVLLMLISPLSWACTMTFQFRNPNFGGNPNNGAFLLNSAQAQNSYKDPENLYFQSSYNDDFGIETPSALDNFTQAIQSQILGGLLSNINTGKPGRMVTNDYIVDIANRDGQLQLNVTDRKTGQTSTIQVSGLQNNSTDFSAWSHPQFEK

SEQ ID NO: 60 - protein, 155 aa, Artificial Sequence
  a CsgF sequence with a signal sequence, a TEV protease cleavage site (ENLYFQS) inserted between residues 45 and 46 of sequence of the mature protein, and a His10 tag at the C-terminus
MRVKHAVVLLMLISPLSWAGTMTFQFRNPNFGGNPNNGAFLLNSAQAQNSYKDPSYNDDFGIETENLYFQSPSALDNFTQAIQSQILGGLLSNINTGKPGRMVTNDYIVDIANRDGQLQLNVTDRKTGQTSTIQVSGLQNNSTDFHHHHHHHHHH

SEQ ID NO: 61 - protein, 155 aa, Artificial Sequence
  a CsgF sequence with a signal sequence, a TEV protease cleavage site (ENLYFQS) inserted between residues 35 and 36 of sequence of the mature protein, and a His10 tag at the C-terminus
MRVKHAVVLLMLISPLSWAGTMTFQFRNPNFGGNPNNGAFLLNSAQAQNSYKDPENLYFQSSYNDDFGIETPSALDNFTQAIQSQILGGLLSNINTGKPGRMVTNDYIVDIANRDGQLQLNVTDRKTGQTSTIQVSGLQNNSTDFHHHHHHHHHH

SEQ ID NO: 62 - protein, 155 aa, Artificial Sequence
  a CsgF sequence with a signal sequence, a TEV protease cleavage site (ENLYFQS) inserted between residues 30 and 31 of sequence of the mature protein, and a His10 tag at the C-terminus.
MRVKHAVVLLMLISPLSWAGTMTFQFRNPNFGGNPNNGAFLLNSAQAQNENLYFQSSYKDPSYNDDFGIETPSALDNFTQAIQSQILGGLLSNINTGKPGRMVTNDYIVDIANRDGQLQLNVTDRKTGQTSTIQVSGLQNNSTDFHHHHHHHHHH

SEQ ID NO: 63 - protein, 149 aa, Artificial Sequence
  a CsgF sequence with a signal sequence, a TEV protease cleavage site (ENLYFQS) inserted between residues 45 and 51 of sequence of the mature protein, and a His10 tag at the C-terminus
MRVKHAVVLLMLISPLSWAGTMTFQFRNPNFGGNPNNGAFLLNSAQAQNSYKDPSYNDDFGIETENLYFQSFTQAIQSQILGGLLSNINTGKPGRMVTNDYIVDIANRDGQLQLNVTDRKTGQTSTIQVSGLQNNSTDFHHHHHHHHHH

SEQ ID NO: 64 - protein, 149 aa, Artificial Sequence
  a CsgF sequence with a signal sequence, a TEV protease cleavage site (ENLYFQS) inserted between residues 30 and 37 of sequence of the mature protein, and a His10 tag at the C-terminus
MRVKHAVVLLMLISPLSWAGTMTFQFRNPNFGGNPNNGAFLLNSAQAQNENLYFQSYNDDFGIETPSALDNFTQAIQSQILGGLLSNINTGKPGRMVTNDYIVDIANRDGQLQLNVTDRKTGQTSTIQVSGLQNNSTDFHHHHHHHHHH

SEQ ID NO: 65 - protein, 155 aa, Artificial Sequence
  a CsgF sequence with a signal sequence, a HCV C3 protease cleavage site (LEVLFQGP) inserted between residues 34 and 36 of sequence of the mature protein, and a His10 tag at the C-terminus
MRVKHAVVLLMLISPLSWACTMTFQFRNPNFGGNPNNGAFLLNSAQAQNSYKDLEVLFQGPSYNDDFGIETPSALDNFTQAIQSQILGGLLSNINTGKPGRMVTNDYIVDIANRDGQLQLNVTDRKTGQTSTIQVSGLQNNSTDFSAWSHPQFEK

SEQ ID NO: 66 - protein, 156 aa, Artificial Sequence
  a CsgF sequence with a signal sequence, a HCV C3 protease cleavage site (LEVLFQGP) inserted between residues 42 and 43 of sequence of the mature protein, and a His10 tag at the C-terminus
MRVKHAVVLLMLISPLSWACTMTFQFRNPNFGGNPNNGAFLLNSAQAQNSYKDPSYNDDFGILEVLFQGPETPSALDNFTQAIQSQILGGLLSNINTGKPGRMVTNDYIVDIANRDGQLQLNVTDRKTGQTSTIQVSGLQNNSTDFSAWSHPQFEK

SEQ ID NO: 67 - protein, 148 aa, Artificial Sequence
  a CsgF sequence with a signal sequence, a HCV C3 protease cleavage site (LEVLFQGP) inserted between residues 38 and 47 of sequence of the mature protein, and a His10 tag at the C-terminus
MRVKHAVVLLMLISPLSWACTMTFQFRNPNFGGNPNNGAFLLNSAQAQNSYKDPSYNLEVLFQGPSALDNFTQAIQSQILGGLLSNINTGKPGRMVTNDYIVDIANRDGQLQLNVTDRKTGQTSTIQVSGLQNNSTDFSAWSHPQFEK

SEQ ID NO: 68 - protein, 248 aa, Citrobacter koseri
MPRAQSYKDLTHLPMPTGKIFVSVYNIQDETGQFKPYPASNFSTAVPQSATAMLVTALKDSRWFIPLERQGLQNLLNERKIIRAAQENGTVAINNRIPLQSLTAANIMVEGSIIGYESNVKSGGVGARYFGIGADTQYQLDQIAVNLRVVNVSTGEILSSVNTSKTILSYEVQAGVFRFIDYQRLLEGEIGYTSNEPVMLCLMSAIETGVIFLINDGIDRGLWDLQNKAERQNDILVKYRHMSVPPES

SEQ ID NO: 69 - protein, 223 aa, Salmonella enterica
CLTAPPKQAAKPTLMPRAQSYKDLTHLPAPTGKIFVSVYNIQDETGQFKPYPASNFSTAVPQSATAMLVTALKDSRWFIPLERQGLQNLLNERKIIRAAQENGTVAMNNRIPLQSLTAANIMVEGSIIGYESNVKSGGVGARYFGIGADTQYQLDQIAVNLRVVNVSTGEILSSVNTSKTILSYEVQAGVFRFIDYQRLLEGEIGYTSNEPVMLCLMSAIETG

SEQ ID NO: 70 - protein, 262 aa, Citrobacter amalonaticus
CLTAPPKEAAKPTLMPRAQSYKDLTHLPIPTGKIFVSVYNIQDETGQFKPYPASNFSTAVPQSATAMLVTALKDSRWFVPLERQGLQNLLNERKIIRAAQENGTVAINNRIPLQSLTAANIMVEGSIIGYESNVKSGGVGARYFGIGADTQYQLDQIAVNLRVVNVSTGEILSSVNTSKTILSYEVQAGVFRFIDYQRLLEGEIGYTSNEPVMLCLMSAIETGVIFLINDGIDRGLWDLQNKADRQNDILVKYRHMSVPPES

SEQ ID NO: 71 - protein, 262 aa, Citrobacter rodentium
CLTTPPKEAAKPTLMPRAQSYKDLTHLPVPTGKIFVSVYNIQDETGQFKPYPASNFSTAVPQSATAMLVTALKDSRWFIPLERQGLQNLLNERKIIRAAQENGTVAINNRIPLPSLTAANIMVEGSIIGYESNVKSGGAGARYFGIGADTQYQLDQIAVNLRVVNVSTGEILSSVNTSKTILSYEVQAGVFRFIDYQRLLEGEIGYTSNEPVMLCLMSAIETGVIFLINDGIDRGLWDLQNKADRQNDILVKYRQMSVPPES

SEQ ID NO: 72 - protein, 262 aa, Enterobacter asburiae
CLTAPPKEAAKPTLMPRAQSYRDLTHLPAPTGKIFVSVYNIQDETGQFKPYPASNFSTAVPQSATAMLVTALKDSHWFIPLERQGLQNLLNERKIIRAAQENGTVANNNRMPLQSLAAANVMIEGSIIGYESNVKSGGVGARYFGIGADTQYQLDQIAVNLRVVNVSTGEVLSSVNTSKTILSYEVQAGVFRFIDYQRLLEGEIGYTSNEPVMMCLMSAIETGVIFLINDGIDRGLWDLQNKADAQNPVLVKYRDMSVPPES

SEQ ID NO: 73 - protein, 262 aa, Yokenella regensburgei
CLTAPPKEAAKPTLMPRAQSYRDLTHLPLPSGKVFVSVYNIQDETGQFKPYPASNFSTAVPQSATAMLVTALKDSRWFVPLERQGLQNLLNERKIIRAAQENGTVADNNRIPLQSLTAANVMIEGSIIGYESNVKSGGVGARYFGIGADTQYQLDQIAVNLRVVNVSTGEVLSSVNTSKTILSYEVQAGVFRFVDYQRLLEGEIGYTSNEPVMLCLMSAIETGVIYLINDGIERGLWDLQQKADVDNPILARYRNMSAPPES

SEQ ID NO: 74 - protein, 262 aa, Cronobacter pulveris
CLTAPPKEAAKPTLMPRAQSYRDLTNLPDPKGKLFVSVYNIQDETGQFKPYPASNFSTAVPQSATSMLVTALKDSRWFIPLERQGLQNLLNERKIIRAAQENGTVAENNRMPLQSLVAANVMIEGSIIGYESNVKSGGVGARYFGIGGDTQYQLDQIAVNLRVVNVSTGEVLSSVNTSKTILSYEVQAGVFRFIDYQRLLEGEIGYTANEPVMLCLMSAIETGVIHLINDGINRGLWELKNKGDAKNTILAKYRSMAVPPES

SEQ ID NO: 75 - protein, 262 aa, Rahnella aquatilis
CLTAAPKEAARPTLLPRAPSYTDLTHLPSPQGRIFVSVYNIQDETGQFKPYPACNFSTAVPQSATAMLVSALKDSKWFIPLERQGLQNLLNERKIIRAAQENGSVAINNQRPLSSLVAANILIEGSIIGYESNVKSGGVGARYFGIGASTQYQLDQIAVNLRAVDVNTGEVLSSVNTSKTILSYEVQAGVFRFIDYQRLLEGELGYTTNEPVMLCLMSAIESGVIYLVNDGIERNLWQLQNPSEINSPILQRYKNNIVPAES

SEQ ID NO: 76 - protein, 259 aa, Kluyvera ascorbata
CITSPPKQAAKPTLLPRSQSYQDLTHLPEPQGRLFVSVYNISDETGQFKPYPASNFSTSVPQSATAMLVSALKDSNWFIPLERQGLQNLLNERKIIRAAQENGTVAVNNRTQLPSLVAANILIEGSIIGYESNVKSGGAGARYFGIGASTQYQLDQIAVNLRVVNVSTGEVLSSVNTSKTILSYEFQAGVFRYIDYQRLLEGEVGYTVNEPVMLCLMSAIETGVIYLVNDGISRNLWQLKNASDINSPVLEKYKSIIVP

SEQ ID NO: 77 - protein, 259 aa, Hafnia alvei
CLTAPPKQAAKPTLMPRAQSYQDLTHLPEPAGKLFVSVYNIQDETGQFKPYPASNFSTAVPQSATAMLVSALKDSGWFIPLERQGLQNLLNERKIIRAAQENGTAAVNNQHQLSSLVAANVLVEGSIIGYESNVKSGGAGARFFGIGASTQYQLDQIAVNLRVVDVNTGQVLSSVNTSKTILSYEVQAGVFRYIDYQRLLEGEIGYTTNEPVMLCVMSAIETGVIYLVNDGINRNLWTLKNPQDAKSSVLERYKSTIVP

SEQ ID NO: 78 - protein, 255 aa, Enterobacteriaceae bacterium
CITTPPQEAAKPTLLPRDATYKDLVSLPQPRGKIYVAVYNIQDETGQFQPYPASNFSTSVPQSATAMLVSSLKDSRWFVPLERQGLNNLLNERKIIRAAQQNGTVGDNNASPLPSLYSANVIVEGSIIGYASNVKTGGFGARYFGIGGSTQYQLDQVAVNLRIVNVHTGEVLSSVNTSKTILSYEIQAGVFRFIDYQRLLEGEAGFTTNEPVMTCLMSAIEEGVIHLINDGINKKLWALSNAADINSEVLTRYRK

SEQ ID NO: 79 - protein, 258 aa, Plesiomonas shigelloides
ITEVPKEAAKPTLMPRASTYKDLVALPKPNGKIIVSVYSVQDETGQFKPLPASNFSTAVPQSGNAMLTSALKDSGWFVPLEREGLQNLLNERKIIRAAQENGTVAANNQQPLPSLLSANVVIEGAIIGYDSDIKTGGAGARYFGIGADGKYRVDQVAVNLRAVDVRTGEVLLSVNTSKTILSSELSAGVFRFIEYQRLLELEAGYTTNEPVMMCMMSALEAGVAHLIVEGIRQNLWSLQNPSDINNPIIQRYMKEDVP

SEQ ID NO: 80 - protein, 248 aa, Vibrio fischeri
PETSESPTLMQRGANYIDLISLPKPQGKIFVSVYDFRDQTGQYKPQPNSNFSTAVPQGGTALLTMALLDSEWFYPLERQGLQNLLTERKIIRAAQKKQESISNHGSTLPSLLSANVMIEGGIVAYDSNIKTGGAGARYLGIGGSGQYRADQVTVNIRAVDVRSGKILTSVTTSKTILSYEVSAGAFRFVDYKELLEVELGYTNNEPVNIALMSAIDSAVIHLIVKGVQQGLWRPANLDTRNNPIFKKY

SEQ ID NO: 81 - protein, 248 aa, Aliivibrio logei
PDASESPTLMQRGATYLDLISLPKPQGKIYVSVYDFRDQTGQYKPQPNSNFSTAVPQGGTALLTMALLDSEWFYPLERQGLQNLLTERKIIRAAQKKQESISNHGSTLPSLLSANVMIEGGIVAYDSNIKTGGAGARYLGIGGSGQYRADQVTVNIRAVDVRSGKILTSVTTSKTILSYELSAGAFRFVDYKELLEVELGYTNNEPVNIALMSAIDSAVIHLIVKGIEEGLWRPENQNGKENPIFRKY

SEQ ID NO: 82 - protein, 254 aa, Photobacterium sp.
PETSKEPTLMARGTAYQDLVSLPLPKGKVYVSVYDFRDQTGQYKPQPNSNFSTAVPQGGAALLTTALLDSRWFMPLEREGLQNLLTERKIIRAAQKKDEIPTNHGVHLPSLASANIMVEGGIVAYDTNIQTGGAGARYLGVGASGQYRTDQVTVNIRAVDVRTGRILLSVTTSKTILSKELQTGVFKFVDYKDLLEAELGYTTNEPVNLAVMSAIDAAVVHVIVDGIKTGLWEPLRGEDLQHPIIQEYMNRSKP

SEQ ID NO: 83 - protein, 261 aa, Aeromonas veronii
CATHIGSPVADEKATLMPRSVSYKELISLPKPKGKIVAAVYDFRDQTGQYLPAPASNFSTAVTQGGVAMLSTALWDSQWFVPLEREGLQNLLTERKIVRAAQNKPNVPGNNANQLPSLVAANILIEGGIVAYDSNVRTGGAGAKYFGIGASGEYRVDQVTVNLRAVDIRSGRILNSVTTSKTVMSQQVQAGVFRFVEYKRLLEAEAGFSTNEPVQMCVMSAIESGVIRLIANGVRDNLWQLADQRDIDNPILQEYLQDNAP

SEQ ID NO: 84 - protein, 239 aa, Shewanella sp.
ASSSLMPKGESYYDLINLPAPQGVMLAAVYDFRDQTGQYKPIPSSNFSTAVPQSGTAFLAQALNDSSWFIPVEREGLQNLLTERKIVRAGLKGDANKLPQLNSAQILMEGGIVAYDTNVRTGGAGARYLGIGAATQFRVDTVTVNLRAVDIRTGRLLSSVTTTKSILSKEITAGVFKFIDAQELLESELGYTSNEPVSLCVASAIESAVVHMIADGIWKGAWNLADQASGLRSPVLQKY

SEQ ID NO: 85 - protein, 233 aa, Pseudomonas putida
QDSETPTLTPRASTYYDLINMPRPKGRLMAVVYGFRDQTGQYKPTPASSFSTSVTQGAASMLMDALSASGWFVVLEREGLQNLLTERKIIRASQKKPDVAENIMGELPPLQAANLMLEGGIIAYDTNVRSGGEGARYLGIDISREYRVDQVTVNLRAVDVRTGQVLANVMTSKTIYSVGRSAGVFKFIEFKKLLEAEVGYTTNEPAQLCVLSAIESAVGHLLAQGIEQRLWQV

SEQ ID NO: 86 - protein, 234 aa, Shewanella violacea
MPKSDTYYDLIGLPHPQGSMLAAVYDFRDQTGQYKAIPSSNFSTAVPQSGTAFLAQALNDSSWFVPVEREGLQNLLTERKIVRAGLKGEANQLPQLSSAQILMEGGIVAYDTNIKTGGAGARYLGIGVNSKFRVDTVTVNLRAVDIRTGRLLSSVTTTKSILSKEVSAGVFKFIDAQDLLESELGYTSNEPVSLCVAQAIESAVVHMIADGIWKRAWNLADTASGLNNPVLQKY

SEQ ID NO: 87 - protein, 245 aa, Marinobacterium jannaschii
LTRRMSTYQDLIDMPAPRGKIVTAVYSFRDQSGQYKPAPSSSFSTAVTQGAAAMLVNVLNDSGWFIPLEREGLQNILTERKIIRAALKKDNVPVNNSAGLPSLLAANIMLEGGIVGYDSNIHTGGAGARYFGIGASEKYRVDEVTVNLRAIDIRTGRILHSVLTSKKILSREIRSDVYRFIEFKHLLEMEAGITTNDPAQLCVLSAIESAVAHLIVDGVIKKSWSLADPNELNSPVIQAYQQQRI

SEQ ID NO: 88 - protein, 234 aa, Chryseobacterium oranimense
PSDPERSTMGELTPSTAELRNLPLPNEKIVIGVYKFRDQTGQYKPSENGNNWSTAVPQGTTTILIKALEDSRWFIPIERENIANLLNERQIIRSTRQEYMKDADKNSQSLPPLLYAGILLEGGVISYDSNTMTGGFGARYFGIGASTQYRQDRITIYLRAVSTLNGEILKTVYTSKTILSTSVNGSFFRYIDTERLLEAEVGLTQNEPVQLAVTEAIEKAVRSLIIEGTRDKIW

SEQ ID NO: 89 - protein, 45 aa, Artificial Sequence
  CsgF peptide
CTMTFQFRNPNFGGNPNNGAFLLNSAQAQNSYKDPSYNDDFGIET

SEQ ID NO: 90 - protein, 29 aa, Artificial Sequence
  CsgF peptide
CTMTFQFRNPNFGGNPNNGAFLLNSAQAQ

SEQ ID NO: 91 - protein, 35 aa, Artificial Sequence
  CsgF peptide
CTMTFQFRNPNFGGNPNNGAFLLNSAQAQNSYKDP

SEQ ID NO: 92 - protein, 35 aa, Artificial Sequence
  CsgF peptide
GTMTFQFRNPNFGGNPSNGAFLLNSAQAQNSYKDP

SEQ ID NO: 93 - protein, 35 aa, Artificial Sequence
  CsgF peptide
CTMTFQFRNPNFGGNPNNGAFLLNSAQAQNSYKYP

SEQ ID NO: 94 - protein, 45 aa, Artificial Sequence
  CsgF peptide
GTMTFQFRNPNFGGNPSNGAFLLNSAQAQNSYKDPSYNDDFGIET

SEQ ID NO: 95 - protein, 35 aa, Artificial Sequence
  CsgF peptide
CTMTFQFRNPNFGGNPSNGAFLLNSAQAQNSYKYP

SEQ ID NO: 96 - protein, 39 aa, Artificial Sequence
  CsgF peptide
CTMTFQFRNPNFGGNPNNGAFLLNSAQAQHHHHHHHHHH

SEQ ID NO: 97 - protein, 45 aa, Artificial Sequence
  CsgF peptide
CTMTFQFRNPNFGGNPNNGAFLLNSAQAQNSYKDPHHHHHHHHHH

SEQ ID NO: 98 - protein, 35 aa, Artificial Sequence
  CsgF peptide
GTMTFQFRNPNFGGNPSNGAFLLNSAQAQNSYKYP

SEQ ID NO: 99 - protein, 35 aa, Artificial Sequence
  CsgF peptide
GTMTFQFRNPNFGGNPSNGAFLLNSAQAQNSYKNP

SEQ ID NO: 100 - protein, 35 aa, Artificial Sequence
  CsgF peptide
GTMCFQFRNPNFGGNPSNGAFLLNSAQAQNSYKDP

SEQ ID NO: 101 - protein, 35 aa, Artificial Sequence
  CsgF peptide
GTMCFQFRNPNFGGNPSNGAFLLNSAQAQNSYKYP

SEQ ID NO: 102 - protein, 35 aa, Artificial Sequence
  CsgF peptide
GTMCFQFRNPNFGGNPSNGAFLLNSAQAQNSYKNP

SEQ ID NO: 103 - protein, 35 aa, Artificial Sequence
  CsgF peptide
CTMCFQFRNPNFGGNPSNGAFLLNSAQAQNSYKDP

SEQ ID NO: 104 - protein, 35 aa, Artificial Sequence
  CsgF peptide
CTMCFQFRNPNFGGNPSNGAFLLNSAQAQNSYKNP

SEQ ID NO: 105 - protein, 35 aa, Artificial Sequence
  CsgF peptide
CTMCFQFRNPNFGGNPSNGAFLLNSAQAQNSYKYP

SEQ ID NO: 106 - protein, 35 aa, Artificial Sequence
  CsgF peptide
GTMTFQFRNPNFGGNPVNGAFLLNSAQAQNSYKDP

SEQ ID NO: 107 - protein, 35 aa, Artificial Sequence
  CsgF peptide
GTMTFQFRNPNFGGNPANGAFLLNSAQAQNSYKDP

SEQ ID NO: 108 - protein, 35 aa, Artificial Sequence
  CsgF peptide
GTMTFQFRNPNFGGNPFNGAFLLNSAQAQNSYKDP

SEQ ID NO: 109 - protein, 30 aa, Artificial Sequence
  CsgF peptide
GTMTFQFRNPNFGGNPSNGAFLLNSAQAQN

SEQ ID NO: 110 - protein, 30 aa, Artificial Sequence
  CsgF peptide
GTMTFQFRNPNFGGNPVNGAFLLNSAQAQN

SEQ ID NO: 111 - protein, 30 aa, Artificial Sequence
  CsgF peptide
GTMTFQFRNPNFGGNPANGAFLLNSAQAQN

SEQ ID NO: 112 - protein, 30 aa, Artificial Sequence
  CsgF peptide
GTMTFQFRNPNFGGNPFNGAFLLNSAQAQN

SEQ ID NO: 113 - protein, 35 aa, Artificial Sequence
  CsgF peptide
GTMTFQFRNPNFGGNPVNGAFLLNSAQAQNSYKYP

SEQ ID NO: 114 - protein, 35 aa, Artificial Sequence
  CsgF peptide
GTMTFQFRNPNFGGNPANGAFLLNSAQAQNSYKYP

SEQ ID NO: 115 - protein, 35 aa, Artificial Sequence
  CsgF peptide
GTMTFQFRNPNFGGNPFNGAFLLNSAQAQNSYKYP

SEQ ID NO: 116 - protein, 35 aa, Artificial Sequence
  CsgF peptide
GTMTFQFRNPNFGGNPSNGQFLLNSAQAQNSYKDP

SEQ ID NO: 117 - protein, 14 aa, Artificial Sequence
  CsgF peptide
GTMTFQFRHHHHHH

SEQ ID NO: 118 - protein, 25 aa, Artificial Sequence
  CsgF peptide
GTMTFQFRNPNFGGNPNNGHHHHHH

SEQ ID NO: 119 - protein, 35 aa, Artificial Sequence
  CsgF peptide
GTMTFQFRNPNFGGNPNNGAFLLNSAQAQHHHHHH

SEQ ID NO: 120 - protein, 51 aa, Artificial Sequence
  CsgF peptide
GTMTFQFRNPNFGGNPNNGAFLLNSAQAQNSYKDPSYNDDFGIETHHHHHH